European Patent Application EP 4 155 392 A1, published March 29, 2023. Title: APPLICATION OF TGF-β INHIBITOR IN INDUCING NEURAL STEM CELLS AND ORGANOID FORMATION. Applicant: IREGENE THERAPEUTICS LTD. Application EP21808346.7. The sequence listing filed with the application follows.

SEQUENCE LISTING (24 sequences)

SEQ ID NO: 1 - DNA, 21 bp, Artificial Sequence
  Artificial Sequence
catgcaggttgacaccgttgg

SEQ ID NO: 2 - DNA, 24 bp, Artificial Sequence
  Artificial Sequence
atggattctcggcagactgattca

SEQ ID NO: 3 - DNA, 19 bp, Artificial Sequence
  Artificial Sequence
tctttgcttgggaaatccg

SEQ ID NO: 4 - DNA, 21 bp, Artificial Sequence
  Artificial Sequence
ctgcccgttcaacatccttag

SEQ ID NO: 5 - DNA, 23 bp, Artificial Sequence
  Artificial Sequence
ggaagcgaatcaatggactctgg

SEQ ID NO: 6 - DNA, 22 bp, Artificial Sequence
  Artificial Sequence
gcatcgacatctgtaccagacc

SEQ ID NO: 7 - DNA, 22 bp, Artificial Sequence
  Artificial Sequence
tcaagatgtccctcagcctgga

SEQ ID NO: 8 - DNA, 23 bp, Artificial Sequence
  Artificial Sequence
tggcacaggtgtctcaagggtag

SEQ ID NO: 9 - DNA, 20 bp, Artificial Sequence
  Artificial Sequence
tccctggagaagagctacga

SEQ ID NO: 10 - DNA, 20 bp, Artificial Sequence
  Artificial Sequence
agcactgtgttggcgtacag

SEQ ID NO: 11 - DNA, 23 bp, Artificial Sequence
  Artificial Sequence
caagcagagcggatgtctcagat

SEQ ID NO: 12 - DNA, 24 bp, Artificial Sequence
  Artificial Sequence
aattgtagaggaggcgaacaggag

SEQ ID NO: 13 - DNA, 22 bp, Artificial Sequence
  Artificial Sequence
tgtggtggtgccttctggagag

SEQ ID NO: 14 - DNA, 23 bp, Artificial Sequence
  Artificial Sequence
actgcttgcagcctgagtgtaac

SEQ ID NO: 15 - DNA, 22 bp, Artificial Sequence
  Artificial Sequence
cgcttcatctcagtgggctacg

SEQ ID NO: 16 - DNA, 23 bp, Artificial Sequence
  Artificial Sequence
ccgtcctcgctctggttgtagta

SEQ ID NO: 17 - DNA, 20 bp, Artificial Sequence
  Artificial Sequence
aacctgctccgccgctacaa

SEQ ID NO: 18 - DNA, 24 bp, Artificial Sequence
  Artificial Sequence
tcctctgcatattcctctgcctca

SEQ ID NO: 19 - DNA, 24 bp, Artificial Sequence
  Artificial Sequence
tcatctgtggagtgggcatcttca

SEQ ID NO: 20 - DNA, 24 bp, Artificial Sequence
  Artificial Sequence
agcaacttcttggcagcagtatcc

SEQ ID NO: 21 - DNA, 24 bp, Artificial Sequence
  Artificial Sequence
ggacaatgacgttgaaacgcagca

SEQ ID NO: 22 - DNA, 24 bp, Artificial Sequence
  Artificial Sequence
aaggtcgtaagcggtttggctaga

SEQ ID NO: 23 - DNA, 22 bp, Artificial Sequence
  Artificial Sequence
ctggagaggaagattgagtcgc

SEQ ID NO: 24 - DNA, 22 bp, Artificial Sequence
  Artificial Sequence
acgtcaagctccacatggacct